European Patent Application EP 4 501 349 A1, published February 5, 2025. Title: Botulinum toxin protein composition, method for preparing same, and use thereof. Applicant: Chongqing Claruvis Pharmaceutical Co., LTD. Application WO PCT/CN2023/085106, filed March 30, 2023. The sequence listing filed with the application follows.

SEQUENCE LISTING (22 sequences)

SEQ ID NO: 1 - DNA, 654 bp, synthetic construct
  source 1..654: mol_type = other DNA
atgtcccctatactaggttattggaaaattaagggccttgtgcaacccactcgacttcttttggaatatcttgaagaaaaatatgaagagcatttgtatgagcgcgatgaaggtgataaatggcgaaacaaaaagtttgaattgggtttggagtttcccaatcttccttattatattgatggtgatgttaaattaacacagtctatggccatcatacgttatatagctgacaagcacaacatgttgggtggttgtccaaaagagcgtgcagagatttcaatgcttgaaggagcggttttggatattagatacggtgtttcgagaattgcatatagtaaagactttgaaactctcaaagttgattttcttagcaagctacctgaaatgctgaaaatgttcgaagatcgtttatgtcataaaacatatttaaatggtgatcatgtaacccatcctgacttcatgttgtatgacgctcttgatgttgttttatacatggacccaatgtgcctggatgcgttcccaaaattagtttgttttaaaaaacgtattgaagctatcccacaaattgataagtacttgaaatccagcaagtatatagcatggcctttgcagggctggcaagccacgtttggtggtggcgaccatcctccaaaa

SEQ ID NO: 2 - protein, 218 aa, synthetic construct
MSPILGYWKIKGLVQPTRLLLEYLEEKYEEHLYERDEGDKWRNKKFELGLEFPNLPYYIDGDVKLTQSMAIIRYIADKHNMLGGCPKERAEISMLEGAVLDIRYGVSRIAYSKDFETLKVDFLSKLPEMLKMFEDRLCHKTYLNGDHVTHPDFMLYDALDVVLYMDPMCLDAFPKLVCFKKRIEAIPQIDKYLKSSKYIAWPLQGWQATFGGGDHPPK

SEQ ID NO: 3 - DNA, 24 bp, synthetic construct
  source 1..24: mol_type = other DNA
ctggaagttctgttccaggggccc

SEQ ID NO: 4 - protein, 8 aa, synthetic construct
LEVLFQGP

SEQ ID NO: 5 - skipped

SEQ ID NO: 6 - DNA, 3882 bp, synthetic construct
  source 1..3882: mol_type = other DNA
atgcctttcgttaacaaacagtttaactataaggacccggttaacggtgtggatattgcatacattaagatccctaacgctggtcagatgcagccggtgaaagcattcaagatccacaataagatttgggtgatcccggaacgcgatacctttaccaacccggaagaaggcgatctgaacccccctccggaggccaagcaagttcccgttagctattacgacagtacctatttaagcaccgataatgagaaagataactatctgaagggtgttaccaaactgttcgagcgcatctacagcacagacttaggccgcatgctgctgaccagtatcgttcgtggtattccgttctggggcggcagtaccatcgacaccgagctgaaagtgatcgacaccaattgcattaacgtgatccagcccgatggcagctatcgtagcgaagagctgaatctggttatcatcggccctagtgccgacattattcaattcgagtgtaaaagcttcggccatgaggtgctgaatttaacccgtaatggctatggcagtacccagtacatccgcttcagcccggattttaccttcggcttcgaggaatctttagaagtggataccaatccgctgctgggcgccggcaaatttgcaacagaccccgctgttactttagcccatgagctgattcatgctggtcatcgtctgtacggcatcgccattaacccgaaccgtgtgtttaaggttaacaccaacgcctattatgaaatgagtggtttagaggtgagcttcgaggagctgcgtacctttggtggccatgatgccaagttcatcgatagtctgcaagaaaacgagtttcgtctgtattattacaacaagttcaaagatatcgcaagcaccttaaataaagccaagagcatcgttggcaccaccgcctctttacaatatatgaaaaacgttttcaaggagaaatatctgctgagcgaggacaccagtggtaaatttagtgttgacaaactgaagttcgataaactgtataagatgctgaccgagatctataccgaagacaatttcgtgaaattttttaaagttctgaatcgcaaaacatatttaaacttcgacaaagcagtgtttaaaatcaacatcgttccgaaggttaattacacaatctacgatggcttcaatttacgcaacaccaatttagccgcaaacttcaacggccaaaataccgagatcaataacatgaatttcaccaaactgaaaaactttactggtttatttgagttctacaaactgctgtgcgtgcgtggcattatcaccagtttagaagtgctgtttcaaggtccggccttaaacgatctgtgtattaaagttaacaattgggatctgtttttcagccctagcgaggacaattttaccaacgatttaaacaaaggcgaggagatcaccagcgataccaatattgaggccgcagaggagaatatcagtctggatttaatccagcaatattatctgacctttaattttgacaatgagccggagaacattagtatcgaaaatttaagtagcgacatcattggtcagctggagctgatgccgaacattgagcgcttcccgaatggcaaaaagtatgaattagataagtacaccatgtttcactatttacgcgcccaagaatttgaacacggtaaaagccgtattgccttaaccaacagcgtgaatgaagcactgctgaacccgagccgcgtgtatacctttttcagtagtgactatgttaagaaggtgaataaggccaccgaagccgccatgttcttaggctgggtggagcagctggtgtatgatttcaccgatgagaccagcgaggtgagcaccacagataaaatcgcagatattacaattattattccgtacatcggcccggctttaaatatcggtaacatgctgtacaaagatgatttcgtgggcgctttaatctttagcggtgccgttattctgttagaattcattcccgaaattgcaatcccggtgctgggcacctttgctttagttagctatatcgcaaataaagtgttaaccgttcagaccattgacaatgctttaagcaagcgtaatgaaaagtgggatgaggtttataaatacatcgttacaaattggttagccaaagtgaacacccagattgatttaatccgtaagaaaatgaaagaagccttagagaatcaagctgaggccacaaaagcaattatcaattaccagtacaatcagtataccgaagaagaaaagaacaatatcaactttaatattgatgatttaagcagcaagctgaacgaaagcattaataaagccatgattaatattaacaagtttttaaaccagtgcagcgtgagctatttaatgaacagcatgatcccttacggtgtgaagcgtctggaagatttcgatgcctctttaaaagacgcactgttaaagtatatttatgacaatcgcggcacactgatcggtcaagttgatcgtctgaaagataaagttaataacacattaagcacagacattcctttccagctgagtaaatacgtggacaatcaacgtctgctgagcacctttaccgaatacattaaaaacattattaacaccagcattctgaatttacgctacgagagcaaccatttaattgatctgagccgttacgccagcaagatcaatatcggtagcaaggttaacttcgacccgattgacaaaaaccagatccagttattcaatttagagagtagtaagattgaggttattttaaaaaacgccatcgtttataacagcatgtacgaaaattttagcacaagcttttggattcgtatcccgaagtatttcaatagcatctctttaaataatgaatacacaatcattaattgcatggaaaacaacagcggctggaaggtgtctttaaactacggtgagatcatctggactttacaagatacccaagaaatcaagcagcgcgttgtgttcaaatatagtcagatgatcaacattagtgactatattaaccgctggatttttgtgaccatcacaaataaccgtttaaacaacagcaaaatttatattaacggtcgtctgattgaccagaagccgattagcaatttaggtaatatccatgccagcaacaacattatgttcaaactggatggttgtcgcgatacccatcgctacatctggattaagtactttaacttattcgacaaagaactgaatgaaaaggagatcaaggacttatatgataatcaaagcaatagcggcattttaaaagacttttggggtgactatctgcagtatgacaaaccttactatatgctgaacttatatgacccgaacaaatacgttgacgtgaacaatgtgggtattcgtggctacatgtatctgaaaggcccgcgcggcagtgttatgaccacaaatatttatttaaacagctctttatatcgtggcaccaagtttatcatcaagaagtacgcaagcggcaataaagacaatattgtgcgtaacaacgatcgtgtgtacatcaacgttgtggtgaagaacaaagagtatcgtttagccaccaatgccagccaagctggtgtggaaaaaattttaagcgcactggagatccccgatgtgggcaatttaagtcaagttgttgtgatgaaaagtaagaatgatcaaggcatcaccaacaaatgtaagatgaatttacaagacaataacggcaatgacattggttttattggtttccatcagttcaacaatatcgcaaagctggtggccagcaactggtacaaccgtcagatcgaacgtagcagccgtactttaggttgcagctgggaatttattccggtggatgatggttggggtgagcgccctttataa

SEQ ID NO: 7 - protein, 1293 aa, synthetic construct
MPFVNKQFNYKDPVNGVDIAYIKIPNAGQMQPVKAFKIHNKIWVIPERDTFTNPEEGDLNPPPEAKQVPVSYYDSTYLSTDNEKDNYLKGVTKLFERIYSTDLGRMLLTSIVRGIPFWGGSTIDTELKVIDTNCINVIQPDGSYRSEELNLVIIGPSADIIQFECKSFGHEVLNLTRNGYGSTQYIRFSPDFTFGFEESLEVDTNPLLGAGKFATDPAVTLAHELIHAGHRLYGIAINPNRVFKVNTNAYYEMSGLEVSFEELRTFGGHDAKFIDSLQENEFRLYYYNKFKDIASTLNKAKSIVGTTASLQYMKNVFKEKYLLSEDTSGKFSVDKLKFDKLYKMLTEIYTEDNFVKFFKVLNRKTYLNFDKAVFKINIVPKVNYTIYDGFNLRNTNLAANFNGQNTEINNMNFTKLKNFTGLFEFYKLLCVRGIITSLEVLFQGPALNDLCIKVNNWDLFFSPSEDNFTNDLNKGEEITSDTNIEAAEENISLDLIQQYYLTFNFDNEPENISIENLSSDIIGQLELMPNIERFPNGKKYELDKYTMFHYLRAQEFEHGKSRIALTNSVNEALLNPSRVYTFFSSDYVKKVNKATEAAMFLGWVEQLVYDFTDETSEVSTTDKIADITIIIPYIGPALNIGNMLYKDDFVGALIFSGAVILLEFIPEIAIPVLGTFALVSYIANKVLTVQTIDNALSKRNEKWDEVYKYIVTNWLAKVNTQIDLIRKKMKEALENQAEATKAIINYQYNQYTEEEKNNINFNIDDLSSKLNESINKAMININKFLNQCSVSYLMNSMIPYGVKRLEDFDASLKDALLKYIYDNRGTLIGQVDRLKDKVNNTLSTDIPFQLSKYVDNQRLLSTFTEYIKNIINTSILNLRYESNHLIDLSRYASKINIGSKVNFDPIDKNQIQLFNLESSKIEVILKNAIVYNSMYENFSTSFWIRIPKYFNSISLNNEYTIINCMENNSGWKVSLNYGEIIWTLQDTQEIKQRVVFKYSQMINISDYINRWIFVTITNNRLNNSKIYINGRLIDQKPISNLGNIHASNNIMFKLDGCRDTHRYIWIKYFNLFDKELNEKEIKDLYDNQSNSGILKDFWGDYLQYDKPYYMLNLYDPNKYVDVNNVGIRGYMYLKGPRGSVMTTNIYLNSSLYRGTKFIIKKYASGNKDNIVRNNDRVYINVVVKNKEYRLATNASQAGVEKILSALEIPDVGNLSQVVVMKSKNDQGITNKCKMNLQDNNGNDIGFIGFHQFNNIAKLVASNWYNRQIERSSRTLGCSWEFIPVDDGWGERPL

SEQ ID NO: 8 - DNA, 24 bp, synthetic construct
  source 1..24: mol_type = other DNA
ttagaagtgctgtttcaaggtccg

SEQ ID NO: 9 - protein, 8 aa, synthetic construct
LEVLFQGP

SEQ ID NO: 10 - DNA, 4575 bp, synthetic construct
  source 1..4575: mol_type = other DNA
atgtcccctatactaggttattggaaaattaagggccttgtgcaacccactcgacttcttttggaatatcttgaagaaaaatatgaagagcatttgtatgagcgcgatgaaggtgataaatggcgaaacaaaaagtttgaattgggtttggagtttcccaatcttccttattatattgatggtgatgttaaattaacacagtctatggccatcatacgttatatagctgacaagcacaacatgttgggtggttgtccaaaagagcgtgcagagatttcaatgcttgaaggagcggttttggatattagatacggtgtttcgagaattgcatatagtaaagactttgaaactctcaaagttgattttcttagcaagctacctgaaatgctgaaaatgttcgaagatcgtttatgtcataaaacatatttaaatggtgatcatgtaacccatcctgacttcatgttgtatgacgctcttgatgttgttttatacatggacccaatgtgcctggatgcgttcccaaaattagtttgttttaaaaaacgtattgaagctatcccacaaattgataagtacttgaaatccagcaagtatatagcatggcctttgcagggctggcaagccacgtttggtggtggcgaccatcctccaaaatcggatctggaagttctgttccaggggcccctgggatccatgcctttcgttaacaaacagtttaactataaggacccggttaacggtgtggatattgcatacattaagatccctaacgctggtcagatgcagccggtgaaagcattcaagatccacaataagatttgggtgatcccggaacgcgatacctttaccaacccggaagaaggcgatctgaacccccctccggaggccaagcaagttcccgttagctattacgacagtacctatttaagcaccgataatgagaaagataactatctgaagggtgttaccaaactgttcgagcgcatctacagcacagacttaggccgcatgctgctgaccagtatcgttcgtggtattccgttctggggcggcagtaccatcgacaccgagctgaaagtgatcgacaccaattgcattaacgtgatccagcccgatggcagctatcgtagcgaagagctgaatctggttatcatcggccctagtgccgacattattcaattcgagtgtaaaagcttcggccatgaggtgctgaatttaacccgtaatggctatggcagtacccagtacatccgcttcagcccggattttaccttcggcttcgaggaatctttagaagtggataccaatccgctgctgggcgccggcaaatttgcaacagaccccgctgttactttagcccatgagctgattcatgctggtcatcgtctgtacggcatcgccattaacccgaaccgtgtgtttaaggttaacaccaacgcctattatgaaatgagtggtttagaggtgagcttcgaggagctgcgtacctttggtggccatgatgccaagttcatcgatagtctgcaagaaaacgagtttcgtctgtattattacaacaagttcaaagatatcgcaagcaccttaaataaagccaagagcatcgttggcaccaccgcctctttacaatatatgaaaaacgttttcaaggagaaatatctgctgagcgaggacaccagtggtaaatttagtgttgacaaactgaagttcgataaactgtataagatgctgaccgagatctataccgaagacaatttcgtgaaattttttaaagttctgaatcgcaaaacatatttaaacttcgacaaagcagtgtttaaaatcaacatcgttccgaaggttaattacacaatctacgatggcttcaatttacgcaacaccaatttagccgcaaacttcaacggccaaaataccgagatcaataacatgaatttcaccaaactgaaaaactttactggtttatttgagttctacaaactgctgtgcgtgcgtggcattatcaccagtttagaagtgctgtttcaaggtccggccttaaacgatctgtgtattaaagttaacaattgggatctgtttttcagccctagcgaggacaattttaccaacgatttaaacaaaggcgaggagatcaccagcgataccaatattgaggccgcagaggagaatatcagtctggatttaatccagcaatattatctgacctttaattttgacaatgagccggagaacattagtatcgaaaatttaagtagcgacatcattggtcagctggagctgatgccgaacattgagcgcttcccgaatggcaaaaagtatgaattagataagtacaccatgtttcactatttacgcgcccaagaatttgaacacggtaaaagccgtattgccttaaccaacagcgtgaatgaagcactgctgaacccgagccgcgtgtatacctttttcagtagtgactatgttaagaaggtgaataaggccaccgaagccgccatgttcttaggctgggtggagcagctggtgtatgatttcaccgatgagaccagcgaggtgagcaccacagataaaatcgcagatattacaattattattccgtacatcggcccggctttaaatatcggtaacatgctgtacaaagatgatttcgtgggcgctttaatctttagcggtgccgttattctgttagaattcattcccgaaattgcaatcccggtgctgggcacctttgctttagttagctatatcgcaaataaagtgttaaccgttcagaccattgacaatgctttaagcaagcgtaatgaaaagtgggatgaggtttataaatacatcgttacaaattggttagccaaagtgaacacccagattgatttaatccgtaagaaaatgaaagaagccttagagaatcaagctgaggccacaaaagcaattatcaattaccagtacaatcagtataccgaagaagaaaagaacaatatcaactttaatattgatgatttaagcagcaagctgaacgaaagcattaataaagccatgattaatattaacaagtttttaaaccagtgcagcgtgagctatttaatgaacagcatgatcccttacggtgtgaagcgtctggaagatttcgatgcctctttaaaagacgcactgttaaagtatatttatgacaatcgcggcacactgatcggtcaagttgatcgtctgaaagataaagttaataacacattaagcacagacattcctttccagctgagtaaatacgtggacaatcaacgtctgctgagcacctttaccgaatacattaaaaacattattaacaccagcattctgaatttacgctacgagagcaaccatttaattgatctgagccgttacgccagcaagatcaatatcggtagcaaggttaacttcgacccgattgacaaaaaccagatccagttattcaatttagagagtagtaagattgaggttattttaaaaaacgccatcgtttataacagcatgtacgaaaattttagcacaagcttttggattcgtatcccgaagtatttcaatagcatctctttaaataatgaatacacaatcattaattgcatggaaaacaacagcggctggaaggtgtctttaaactacggtgagatcatctggactttacaagatacccaagaaatcaagcagcgcgttgtgttcaaatatagtcagatgatcaacattagtgactatattaaccgctggatttttgtgaccatcacaaataaccgtttaaacaacagcaaaatttatattaacggtcgtctgattgaccagaagccgattagcaatttaggtaatatccatgccagcaacaacattatgttcaaactggatggttgtcgcgatacccatcgctacatctggattaagtactttaacttattcgacaaagaactgaatgaaaaggagatcaaggacttatatgataatcaaagcaatagcggcattttaaaagacttttggggtgactatctgcagtatgacaaaccttactatatgctgaacttatatgacccgaacaaatacgttgacgtgaacaatgtgggtattcgtggctacatgtatctgaaaggcccgcgcggcagtgttatgaccacaaatatttatttaaacagctctttatatcgtggcaccaagtttatcatcaagaagtacgcaagcggcaataaagacaatattgtgcgtaacaacgatcgtgtgtacatcaacgttgtggtgaagaacaaagagtatcgtttagccaccaatgccagccaagctggtgtggaaaaaattttaagcgcactggagatccccgatgtgggcaatttaagtcaagttgttgtgatgaaaagtaagaatgatcaaggcatcaccaacaaatgtaagatgaatttacaagacaataacggcaatgacattggttttattggtttccatcagttcaacaatatcgcaaagctggtggccagcaactggtacaaccgtcagatcgaacgtagcagccgtactttaggttgcagctgggaatttattccggtggatgatggttggggtgagcgccctttataa

SEQ ID NO: 11 - protein, 1524 aa, synthetic construct
MSPILGYWKIKGLVQPTRLLLEYLEEKYEEHLYERDEGDKWRNKKFELGLEFPNLPYYIDGDVKLTQSMAIIRYIADKHNMLGGCPKERAEISMLEGAVLDIRYGVSRIAYSKDFETLKVDFLSKLPEMLKMFEDRLCHKTYLNGDHVTHPDFMLYDALDVVLYMDPMCLDAFPKLVCFKKRIEAIPQIDKYLKSSKYIAWPLQGWQATFGGGDHPPKSDLEVLFQGPLGSMPFVNKQFNYKDPVNGVDIAYIKIPNAGQMQPVKAFKIHNKIWVIPERDTFTNPEEGDLNPPPEAKQVPVSYYDSTYLSTDNEKDNYLKGVTKLFERIYSTDLGRMLLTSIVRGIPFWGGSTIDTELKVIDTNCINVIQPDGSYRSEELNLVIIGPSADIIQFECKSFGHEVLNLTRNGYGSTQYIRFSPDFTFGFEESLEVDTNPLLGAGKFATDPAVTLAHELIHAGHRLYGIAINPNRVFKVNTNAYYEMSGLEVSFEELRTFGGHDAKFIDSLQENEFRLYYYNKFKDIASTLNKAKSIVGTTASLQYMKNVFKEKYLLSEDTSGKFSVDKLKFDKLYKMLTEIYTEDNFVKFFKVLNRKTYLNFDKAVFKINIVPKVNYTIYDGFNLRNTNLAANFNGQNTEINNMNFTKLKNFTGLFEFYKLLCVRGIITSLEVLFQGPALNDLCIKVNNWDLFFSPSEDNFTNDLNKGEEITSDTNIEAAEENISLDLIQQYYLTFNFDNEPENISIENLSSDIIGQLELMPNIERFPNGKKYELDKYTMFHYLRAQEFEHGKSRIALTNSVNEALLNPSRVYTFFSSDYVKKVNKATEAAMFLGWVEQLVYDFTDETSEVSTTDKIADITIIIPYIGPALNIGNMLYKDDFVGALIFSGAVILLEFIPEIAIPVLGTFALVSYIANKVLTVQTIDNALSKRNEKWDEVYKYIVTNWLAKVNTQIDLIRKKMKEALENQAEATKAIINYQYNQYTEEEKNNINFNIDDLSSKLNESINKAMININKFLNQCSVSYLMNSMIPYGVKRLEDFDASLKDALLKYIYDNRGTLIGQVDRLKDKVNNTLSTDIPFQLSKYVDNQRLLSTFTEYIKNIINTSILNLRYESNHLIDLSRYASKINIGSKVNFDPIDKNQIQLFNLESSKIEVILKNAIVYNSMYENFSTSFWIRIPKYFNSISLNNEYTIINCMENNSGWKVSLNYGEIIWTLQDTQEIKQRVVFKYSQMINISDYINRWIFVTITNNRLNNSKIYINGRLIDQKPISNLGNIHASNNIMFKLDGCRDTHRYIWIKYFNLFDKELNEKEIKDLYDNQSNSGILKDFWGDYLQYDKPYYMLNLYDPNKYVDVNNVGIRGYMYLKGPRGSVMTTNIYLNSSLYRGTKFIIKKYASGNKDNIVRNNDRVYINVVVKNKEYRLATNASQAGVEKILSALEIPDVGNLSQVVVMKSKNDQGITNKCKMNLQDNNGNDIGFIGFHQFNNIAKLVASNWYNRQIERSSRTLGCSWEFIPVDDGWGERPL

SEQ ID NO: 12 - protein, 5 aa, synthetic construct
DDDDK

SEQ ID NO: 13 - protein, 7 aa, synthetic construct
EXXYXQS

SEQ ID NO: 14 - protein, 7 aa, synthetic construct
EXXYXQG

SEQ ID NO: 15 - protein, 11 aa, synthetic construct
LEVLFQGPLGS

SEQ ID NO: 16 - protein, 4 aa, synthetic construct
GGGS

SEQ ID NO: 17 - protein, 5 aa, synthetic construct
GGGGS

SEQ ID NO: 18 - protein, 4 aa, synthetic construct
GSGS

SEQ ID NO: 19 - protein, 5 aa, synthetic construct
GGSGS

SEQ ID NO: 20 - protein, 5 aa, synthetic construct
GSGGS

SEQ ID NO: 21 - protein, 11 aa, synthetic construct
KTKSLDKGYNK

SEQ ID NO: 22 - protein, 5 aa, synthetic construct
GGGSS